European Patent Application EP 4 269 570 A1, published November 1, 2023. Title: Virus vector-producing cells with improved vector-producing ability and methods for production and selection thereof. Applicant: AGC INC. The sequence listing filed with the application follows.

SEQUENCE LISTING (3 sequences)

SEQ ID NO: 1 - RNA, 25 nt, Artificial Sequence
  si-MRE11
gcauccuggugaggaauaacaaggg

SEQ ID NO: 2 - RNA, 21 nt, Artificial Sequence
  si-ISG15
aagaaccuggucccagaggag

SEQ ID NO: 3 - DNA, 21 bp, Artificial Sequence
  si-CD44
ggaccaauuaccauaacuatt